European Patent Application EP 4 640 234 A1, published October 29, 2025. Title: PHARMACEUTICAL COMPOSITION FOR THE PREVENTION OR TREATMENT OF GRAFT-VERSUS-HOST DISEASE CONTAINING GLP-2 DERIVATIVE OR LONG-ACTING CONJUGATE THEREOF. Applicant: HANMI PHARM. CO., LTD. The sequence listing filed with the application follows.

SEQUENCE LISTING (34 sequences)

SEQ ID NO: 1 - protein, 33 aa, Homo sapiens
HADGSFSDEMNTILDNLAARDFINWLIQTKITD

SEQ ID NO: 2 - protein, 34 aa, synthetic construct
  REGION 1..34: note = GLP-2 derivative
  SITE 1: note = X is imidazoacetyldeshistidine
XGDGSFSDEMNTILDNLAARDFINWLIQTKITDC

SEQ ID NO: 3 - protein, 34 aa, synthetic construct
  REGION 1..34: note = GLP-2 derivative
  SITE 1: note = X is imidazoacetyldeshistidine
XGDGSFSDEMNTILDNLAARDFINWLIQTKITDK

SEQ ID NO: 4 - protein, 34 aa, synthetic construct
  REGION 1..34: note = GLP-2 derivative
  SITE 1: note = X is imidazoacetyldeshistidine
XGDGSFSDEMNTILDNLAARDFINWLIQTRITDK

SEQ ID NO: 5 - protein, 34 aa, synthetic construct
  REGION 1..34: note = GLP-2 derivative
  SITE 1: note = X is imidazoacetyldeshistidine
  SITE 34: note = X is 6-azidolysine
XGDGSFSDEMNTILDNLAARDFINWLIQTKITDX

SEQ ID NO: 6 - protein, 34 aa, synthetic construct
  REGION 1..34: note = GLP-2 derivative
  SITE 1: note = X is imidazoacetyldeshistidine
XGDGSFSDEMNTILDNLAARDFINWLIQTRITDC

SEQ ID NO: 7 - protein, 34 aa, synthetic construct
  REGION 1..34: note = GLP-2 derivative
  SITE 1: note = X is imidazoacetyldeshistidine
  SITE 2: note = X is Aib(2-aminoisobutyric acid)
XXDGSFSDEMNTILDNLAARDFINWLIQTKITDC

SEQ ID NO: 8 - protein, 34 aa, synthetic construct
  REGION 1..34: note = GLP-2 derivative
  SITE 2: note = X is Aib(2-aminoisobutyric acid)
HXDGSFSDEMNTILDNLAARDFINWLIQTKITDC

SEQ ID NO: 9 - protein, 34 aa, synthetic construct
  REGION 1..34: note = GLP-2 derivative
  SITE 1: note = X is Histidine, imidazoacetyldeshistidine, desaminohistidine, beta-hydroxyimidazopropionyldeshistidine, N-dimethylhistidine, or beta-carboxyimidazopropionyldeshistidine
  SITE 2: note = X is Alanine, Glycine, or Aib(2-aminoisobutyric acid)
  SITE 30: note = X is Lysine, or Arginine
  SITE 34: note = X is absent, Lysine, Arginine, Glutamine, Histidine, 6-azidolysine, or Cysteine
XXDGSFSDEMNTILDNLAARDFINWLIQTXITDX

SEQ ID NO: 10 - protein, 34 aa, synthetic construct; identical to SEQ ID NO: 9
  REGION 1..34: note = GLP-2 derivative
  SITE 1: note = X is Histidine, imidazoacetyldeshistidine, desaminohistidine, beta-hydroxyimidazopropionyldeshistidine, N-dimethylhistidine, or beta-carboxyimidazopropionyldeshistidine
  SITE 2: note = X is Alanine, Glycine, or Aib(2-aminoisobutyric acid)
  SITE 30: note = X is Lysine, or Arginine
  SITE 34: note = X is any one or more amino acid or any one or more amino acid which is modified

SEQ ID NO: 11 - protein, 12 aa, Homo sapiens
ESKYGPPCPSCP

SEQ ID NO: 12 - protein, 11 aa, synthetic construct
  REGION 1..11: note = Variant of hinge region
ESKYGPPPSCP

SEQ ID NO: 13 - protein, 11 aa, synthetic construct
  REGION 1..11: note = Variant of hinge region
ESKYGPPCPSP

SEQ ID NO: 14 - protein, 10 aa, synthetic construct
  REGION 1..10: note = Variant of hinge region
ESKYGPPCPS

SEQ ID NO: 15 - protein, 10 aa, synthetic construct
  REGION 1..10: note = Variant of hinge region
ESKYGPPCPP

SEQ ID NO: 16 - protein, 8 aa, synthetic construct
  REGION 1..8: note = Variant of hinge region
KYGPPCPS

SEQ ID NO: 17 - protein, 8 aa, synthetic construct
  REGION 1..8: note = Variant of hinge region
ESKYGPPC

SEQ ID NO: 18 - protein, 7 aa, synthetic construct
  REGION 1..7: note = Variant of hinge region
EKYGPPC

SEQ ID NO: 19 - protein, 6 aa, synthetic construct
  REGION 1..6: note = Variant of hinge region
ESPSCP

SEQ ID NO: 20 - protein, 5 aa, synthetic construct
  REGION 1..5: note = Variant of hinge region
EPSCP

SEQ ID NO: 21 - protein, 4 aa, synthetic construct
  REGION 1..4: note = Variant of hinge region
PSCP

SEQ ID NO: 22 - protein, 10 aa, synthetic construct
  REGION 1..10: note = Variant of hinge region
ESKYGPPSCP

SEQ ID NO: 23 - protein, 9 aa, synthetic construct
  REGION 1..9: note = Variant of hinge region
KYGPPPSCP

SEQ ID NO: 24 - protein, 9 aa, synthetic construct
  REGION 1..9: note = Variant of hinge region
ESKYGPSCP

SEQ ID NO: 25 - protein, 8 aa, synthetic construct
  REGION 1..8: note = Variant of hinge region
ESKYGPPC

SEQ ID NO: 26 - protein, 7 aa, synthetic construct
  REGION 1..7: note = Variant of hinge region
KYGPPCP

SEQ ID NO: 27 - protein, 7 aa, synthetic construct
  REGION 1..7: note = Variant of hinge region
ESKPSCP

SEQ ID NO: 28 - protein, 6 aa, synthetic construct
  REGION 1..6: note = Variant of hinge region
ESPSCP

SEQ ID NO: 29 - protein, 4 aa, synthetic construct
  REGION 1..4: note = Variant of hinge region
EPSC

SEQ ID NO: 30 - skipped

SEQ ID NO: 31 - protein, 221 aa, Homo sapiens
PSCPAPEFLGGPSVFLFPPKPKDTLMISRTPEVTCVVVDVSQEDPEVQFNWYVDGVEVHNAKTKPREEQFNSTYRVVSVLTVLHQDWLNGKEYKCKVSNKGLPSSIEKTISKAKGQPREPQVYTLPPSQEEMTKNQVSLTCLVKGFYPSDIAVEWESNGQPENNYKTTPPVLDSDGSFFLYSRLTVDKSRWQEGNVFSCSVMHEALHNHYTQKSLSLSLGK

SEQ ID NO: 32 - protein, 442 aa, Homo sapiens
  REGION 1..442: note = Human Immunoglobulin G4 Fc Fragment (homodimer)
  REGION 1..221: note = Amino acids at position 1 to 221 form one monomer.
  REGION 222..442: note = Amino acids at position 222 to 442 form one monomer.
  DISULFID 3..224: note = Amino acids at position 3 and position 224 form an inter-disulfide bond
  DISULFID 35..95: note = Amino acids at position 35 and position 95 form an intra-chain disulfide bond.
  DISULFID 141..199: note = Amino acids at position 141 and position 199 form an intra-chain disulfide bond.
  DISULFID 256..316: note = Amino acids at position 256 and position 316 form an intra-chain disulfide bond.
  DISULFID 362..420: note = Amino acids at position 362 and position 420 form an intra-chain disulfide bond
PSCPAPEFLGGPSVFLFPPKPKDTLMISRTPEVTCVVVDVSQEDPEVQFNWYVDGVEVHNAKTKPREEQFNSTYRVVSVLTVLHQDWLNGKEYKCKVSNKGLPSSIEKTISKAKGQPREPQVYTLPPSQEEMTKNQVSLTCLVKGFYPSDIAVEWESNGQPENNYKTTPPVLDSDGSFFLYSRLTVDKSRWQEGNVFSCSVMHEALHNHYTQKSLSLSLGKPSCPAPEFLGGPSVFLFPPKPKDTLMISRTPEVTCVVVDVSQEDPEVQFNWYVDGVEVHNAKTKPREEQFNSTYRVVSVLTVLHQDWLNGKEYKCKVSNKGLPSSIEKTISKAKGQPREPQVYTLPPSQEEMTKNQVSLTCLVKGFYPSDIAVEWESNGQPENNYKTTPPVLDSDGSFFLYSRLTVDKSRWQEGNVFSCSVMHEALHNHYTQKSLSLSLGK

SEQ ID NO: 33 - protein, 4 aa, synthetic construct
  source 1..4: note = Linker
GGGS

SEQ ID NO: 34 - protein, 5 aa, synthetic construct
  source 1..5: note = Linker
GGGGS